European Patent Application EP 4 682 891 A2, published January 21, 2026. Title: BIOINFORMATICS SYSTEMS, APPARATUSES, AND METHODS FOR PERFORMING SECONDARY AND/OR TERTIARY PROCESSING. Applicant: Illumina, Inc. The sequence listing filed with the application follows.

SEQUENCE LISTING (3 sequences)

SEQ ID NO: 1 - DNA, 81 bp, synthetic construct
  source 1..81: mol_type = other DNA
tctgctccttatcacacaaggttctaggcacctgatgaggcaaaaaaaaaaaaagaaccctgcaagaatgtgtgcccatgt

SEQ ID NO: 2 - DNA, 11 bp, synthetic construct
  source 1..11: mol_type = other DNA
cgattctaagt

SEQ ID NO: 3 - DNA, 11 bp, synthetic construct
  source 1..11: mol_type = other DNA
cgattgtaagt